European Patent Specification EP 4 021 938 B1, published August 12, 2026. Title: Anti-CR2 Antibodies and Antigen-binding Fragments thereof; and their use in Medical therapy. Applicant: GlaxoSmithKline Intellectual Property Limited, England. The sequence listing filed with the application follows.

SEQUENCE LISTING (74 sequences)

SEQ ID NO: 1 - protein, 1013 aa, Human CR2 sequence
ISCGSPPPILNGRISYYSTPIAVGTVIRYSCSGTFRLIGEKSLLCITKDKVDGTWDKPAPKCEYFNKYSSCPEPIVPGGYKIRGSTPYRHGDSVTFACKTNFSMNGNKSVWCQANNMWGPTRLPTCVSVFPLECPALPMIHNGHHTSENVGSIAPGLSVTYSCESGYLLVGEKIINCLSSGKWSAVPPTCEEARCKSLGRFPNGKVKEPPILRVGVTANFFCDEGYRLQGPPSSRCVIAGQGVAWTKMPVCEEIFCPSPPPILNGRHIGNSLANVSYGSIVTYTCDPDPEEGVNFILIGESTLRCTVDSQKTGTWSGPAPRCELSTSAVQCPHPQILRGRMVSGQKDRYTYNDTVIFACMFGFTLKGSKQIRCNAQGTWEPSAPVCEKECQAPPNILNGQKEDRHMVRFDPGTSIKYSCNPGYVLVGEESIQCTSEGVWTPPVPQCKVAACEATGRQLLTKPQHQFVRPDVNSSCGEGYKLSGSVYQECQGTIPWFMEIRLCKEITCPPPPVIYNGAHTGSSLEDFPYGTTVTYTCNPGPERGVEFSLIGESTIRCTSNDQERGTWSGPAPLCKLSLLAVQCSHVHIANGYKISGKEAPYFYNDTVTFKCYSGFTLKGSSQIRCKADNTWDPEIPVCEKETCQHVRQSLQELPAGSRVELVNTSCQDGYQLTGHAYQMCQDAENGIWFKKIPLCKVIHCHPPPVIVNGKHTGMMAENFLYGNEVSYECDQGFYLLGEKKLQCRSDSKGHGSWSGPSPQCLRSPPVTRCPNPEVKHGYKLNKTHSAYSHNDIVYVDCNPGFIMNGSRVIRCHTDNTWVPGVPTCIKKAFIGCPPPPKTPNGNHTGGNIARFSPGMSILYSCDQGYLLVGEALLLCTHEGTWSQPAPHCKEVNCSSPADMDGIQKGLEPRKMYQYGAVVTLECEDGYMLEGSPQSQCQSDHQWNPPLAVCRSRSLAPVLCGIAAGLILLTFLIVITLYVISKHRARNYYTDTSQKEAFHLEAREVYSVDPYNPAS

SEQ ID NO: 2 - protein, 5 aa, Human CR2 epitope
FNKYS

SEQ ID NO: 3 - protein, 449 aa, Artificial Sequence
  Amino acid sequence identified using molecular biology techniques
QLQLQESGPGLVKPSETLSLTCTVSGGSISSDSYYWGWIRQPPGKGLEWIGSIHYSGSTYYNPPLESRVTISVDTSKNQFSLKLSSVTAADTAVYYCAREGGPRHGWSWGQGTLVTVSSASTKGPSVFPLAPSSKSTSGGTAALGCLVKDYFPEPVTVSWNSGALTSGVHTFPAVLQSSGLYSLSSVVTVPSSSLGTQTYICNVNHKPSNTKVDKKVEPKSCDKTHTCPPCPAPELAGAPSVFLFPPKPKDTLMISRTPEVTCVVVDVSHEDPEVKFNWYVDGVEVHNAKTKPREEQYNSTYRVVSVLTVLHQDWLNGKEYKCKVSNKALPAPIEKTISKAKGQPREPQVYTLPPSRDELTKNQVSLTCLVKGFYPSDIAVEWESNGQPENNYKTTPPVLDSDGSFFLYSKLTVDKSRWQQGNVFSCSVMHEALHNHYTQKSLSLSPGK

SEQ ID NO: 4 - protein, 214 aa, Artificial Sequence
  Amino acid sequence identified using molecular biology techniques
DIQMTQSPSSLSASVGDRVTITCQASQDISEYLNWYQQKPGKAPKLLIYDASNLETGVPSRFSGSGSGTDFTFTISSLQPEDIATYYCQQDSNLPITFGGGTKVEIKRTVAAPSVFIFPPSDEQLKSGTASVVCLLNNFYPREAKVQWKVDNALQSGNSQESVTEQDSKDSTYSLSSTLTLSKADYEKHKVYACEVTHQGLSSPVTKSFNRGEC

SEQ ID NO: 5 - protein, 119 aa, Artificial Sequence
  Amino acid sequence identified using molecular biology techniques
QLQLQESGPGLVKPSETLSLTCTVSGGSISSDSYYWGWIRQPPGKGLEWIGSIHYSGSTYYNPPLESRVTISVDTSKNQFSLKLSSVTAADTAVYYCAREGGPRHGWSWGQGTLVTVSS

SEQ ID NO: 6 - protein, 107 aa, Artificial Sequence
  Amino acid sequence identified using molecular biology techniques
DIQMTQSPSSLSASVGDRVTITCQASQDISEYLNWYQQKPGKAPKLLIYDASNLETGVPSRFSGSGSGTDFTFTISSLQPEDIATYYCQQDSNLPITFGGGTKVEIK

SEQ ID NO: 7 - protein, 7 aa, Artificial Sequence
  Amino acid sequence identified using molecular biology techniques
SDSYYWG

SEQ ID NO: 8 - protein, 16 aa, Artificial Sequence
  Amino acid sequence identified using molecular biology techniques
SIHYSGSTYYNPPLES

SEQ ID NO: 9 - protein, 9 aa, Artificial Sequence
  Amino acid sequence identified using molecular biology techniques
EGGPRHGWS

SEQ ID NO: 10 - protein, 11 aa, Artificial Sequence
  Amino acid sequence identified using molecular biology techniques
QASQDISEYLN

SEQ ID NO: 11 - protein, 7 aa, Artificial Sequence
  Amino acid sequence identified using molecular biology techniques
DASNLET

SEQ ID NO: 12 - protein, 9 aa, Artificial Sequence
  Amino acid sequence identified using molecular biology techniques
QQDSNLPIT

SEQ ID NO: 13 - DNA, 1347 bp, Artificial Sequence
  Amino acid sequence identified using molecular biology techniques
cagctccagctgcaggagagcggcccaggcctggtgaaacccagcgagaccctgagcctgacctgcaccgtgagcggaggcagcatcagctccgacagctactactggggctggattaggcagcctcccggcaagggcctggagtggatcggaagcatccactacagcggcagcacctactacaacccacccctggagagcagggtgaccatcagcgtggacaccagcaagaaccagttcagcctgaagctgagcagcgtcacagcagccgacaccgccgtgtactattgcgccagggagggcggacccaggcacggctggagctggggccagggcaccctggtgaccgtgagcagcgcaagcaccaagggccccagcgtgttccccctggcccccagcagcaagagcaccagcggcggcacagccgccctgggctgcctggtgaaggactacttccccgagcccgtgaccgtgtcctggaacagcggagccctgaccagcggcgtgcacaccttccccgccgtgctgcagagcagcggcctgtacagcctgagcagcgtggtgaccgtgcccagcagcagcctgggcacccagacctacatctgtaacgtgaaccacaagcccagcaacaccaaggtggacaagaaggtggagcccaagagctgtgacaagacccacacctgccccccctgccctgcccccgagctggccggagcccccagcgtgttcctgttcccccccaagcctaaggacaccctgatgatcagcagaacccccgaggtgacctgtgtggtggtggatgtgagccacgaggaccctgaggtgaagttcaactggtacgtggacggcgtggaggtgcacaatgccaagaccaagcccagggaggagcagtacaacagcacctaccgggtggtgtccgtgctgaccgtgctgcaccaggattggctgaacggcaaggagtacaagtgtaaggtgtccaacaaggccctgcctgcccctatcgagaaaaccatcagcaaggccaagggccagcccagagagccccaggtgtacaccctgccccctagcagagatgagctgaccaagaaccaggtgtccctgacctgcctggtgaagggcttctaccccagcgacatcgccgtggagtgggagagcaacggccagcccgagaacaactacaagaccaccccccctgtgctggacagcgatggcagcttcttcctgtacagcaagctgaccgtggacaagagcagatggcagcagggcaacgtgttcagctgctccgtgatgcacgaggccctgcacaatcactacacccagaagagcctgagcctgtcccctggcaag

SEQ ID NO: 14 - DNA, 642 bp, Artificial Sequence
  Amino acid sequence identified using molecular biology techniques
gacatccagatgactcagtccccctctagcctgagcgctagcgtgggcgacagggtgaccatcacctgccaggccagccaggacatcagcgagtacctgaactggtaccagcagaagcccggcaaggcccccaaactgctgatctacgacgcctcaaacctcgagaccggcgtgcctagcaggtttagcggcagcggcagcggcaccgacttcaccttcaccatcagcagcctgcagcccgaggatatcgccacctactactgccagcaggacagcaacctgcccatcaccttcggcggaggcaccaaggtggagattaagcgtacggtggccgcccccagcgtgttcatcttcccccccagcgatgagcagctgaagagcggcaccgccagcgtggtgtgtctgctgaacaacttctacccccgggaggccaaggtgcagtggaaggtggacaatgccctgcagagcggcaacagccaggagagcgtgaccgagcaggacagcaaggactccacctacagcctgagcagcaccctgaccctgagcaaggccgactacgagaagcacaaggtgtacgcctgtgaggtgacccaccagggcctgtccagccccgtgaccaagagcttcaaccggggcgagtgc

SEQ ID NO: 15 - protein, 449 aa, Artificial Sequence
  Amino acid sequence identified using molecular biology techniques
QLQLQESGPGLVKPSETLSLTCTVSGGSISSSSYYWGWIRQPPGKGLEWIGSIHNSGSTYYNPPLKSRVTISVDTSKNQFSLKLSSVTAADTAVYYCAREGGPRHGWSWGQGTLVTVSSASTKGPSVFPLAPSSKSTSGGTAALGCLVKDYFPEPVTVSWNSGALTSGVHTFPAVLQSSGLYSLSSVVTVPSSSLGTQTYICNVNHKPSNTKVDKKVEPKSCDKTHTCPPCPAPELAGAPSVFLFPPKPKDTLMISRTPEVTCVVVDVSHEDPEVKFNWYVDGVEVHNAKTKPREEQYNSTYRVVSVLTVLHQDWLNGKEYKCKVSNKALPAPIEKTISKAKGQPREPQVYTLPPSRDELTKNQVSLTCLVKGFYPSDIAVEWESNGQPENNYKTTPPVLDSDGSFFLYSKLTVDKSRWQQGNVFSCSVMHEALHNHYTQKSLSLSPGK

SEQ ID NO: 16 - protein, 214 aa, Artificial Sequence
  Amino acid sequence identified using molecular biology techniques
DIQMTQSPSSLSASVGDRVTITCQASQDISTFLNWYQQKPGKAPKLLIYDASNLETGVPSRFSGSGSGTDFTFTISSLQPEDIATYYCQQDSILPITFGGGTKVEIKRTVAAPSVFIFPPSDEQLKSGTASVVCLLNNFYPREAKVQWKVDNALQSGNSQESVTEQDSKDSTYSLSSTLTLSKADYEKHKVYACEVTHQGLSSPVTKSFNRGEC

SEQ ID NO: 17 - protein, 119 aa, Artificial Sequence
  Amino acid sequence identified using molecular biology techniques
QLQLQESGPGLVKPSETLSLTCTVSGGSISSSSYYWGWIRQPPGKGLEWIGSIHNSGSTYYNPPLKSRVTISVDTSKNQFSLKLSSVTAADTAVYYCAREGGPRHGWSWGQGTLVTVSS

SEQ ID NO: 18 - protein, 107 aa, Artificial Sequence
  Amino acid sequence identified using molecular biology techniques
DIQMTQSPSSLSASVGDRVTITCQASQDISTFLNWYQQKPGKAPKLLIYDASNLETGVPSRFSGSGSGTDFTFTISSLQPEDIATYYCQQDSILPITFGGGTKVEIK

SEQ ID NO: 19 - protein, 7 aa, Artificial Sequence
  Amino acid sequence identified using molecular biology techniques
SSSYYWG

SEQ ID NO: 20 - protein, 16 aa, Artificial Sequence
  Amino acid sequence identified using molecular biology techniques
SIHNSGSTYYNPPLKS

SEQ ID NO: 21 - protein, 9 aa, Artificial Sequence
  Amino acid sequence identified using molecular biology techniques
EGGPRHGWS

SEQ ID NO: 22 - protein, 11 aa, Artificial Sequence
  Amino acid sequence identified using molecular biology techniques
QASQDISTFLN

SEQ ID NO: 23 - protein, 7 aa, Artificial Sequence
  Amino acid sequence identified using molecular biology techniques
DASNLET

SEQ ID NO: 24 - protein, 9 aa, Artificial Sequence
  Amino acid sequence identified using molecular biology techniques
QQDSILPIT

SEQ ID NO: 25 - DNA, 1347 bp, Nucleic acid sequence encoding '996 heavy chain
cagctccagctgcaggagagcggcccaggcctggtgaaacccagcgagaccctgagcctgacctgcaccgtgagcggaggcagcatcagctccagcagctactactggggctggattaggcagcctcccggcaagggcctggagtggatcggaagcatccacaacagcggcagcacctactacaacccacccctgaagagcagggtgaccatcagcgtggacaccagcaagaaccagttcagcctgaagctgagcagcgtcacagcagccgacaccgccgtgtactattgcgccagggagggcggacccaggcacggctggagctggggccagggcaccctggtgaccgtgagcagcgcaagcaccaagggccccagcgtgttccccctggcccccagcagcaagagcaccagcggcggcacagccgccctgggctgcctggtgaaggactacttccccgagcccgtgaccgtgtcctggaacagcggagccctgaccagcggcgtgcacaccttccccgccgtgctgcagagcagcggcctgtacagcctgagcagcgtggtgaccgtgcccagcagcagcctgggcacccagacctacatctgtaacgtgaaccacaagcccagcaacaccaaggtggacaagaaggtggagcccaagagctgtgacaagacccacacctgccccccctgccctgcccccgagctggccggagcccccagcgtgttcctgttcccccccaagcctaaggacaccctgatgatcagcagaacccccgaggtgacctgtgtggtggtggatgtgagccacgaggaccctgaggtgaagttcaactggtacgtggacggcgtggaggtgcacaatgccaagaccaagcccagggaggagcagtacaacagcacctaccgggtggtgtccgtgctgaccgtgctgcaccaggattggctgaacggcaaggagtacaagtgtaaggtgtccaacaaggccctgcctgcccctatcgagaaaaccatcagcaaggccaagggccagcccagagagccccaggtgtacaccctgccccctagcagagatgagctgaccaagaaccaggtgtccctgacctgcctggtgaagggcttctaccccagcgacatcgccgtggagtgggagagcaacggccagcccgagaacaactacaagaccaccccccctgtgctggacagcgatggcagcttcttcctgtacagcaagctgaccgtggacaagagcagatggcagcagggcaacgtgttcagctgctccgtgatgcacgaggccctgcacaatcactacacccagaagagcctgagcctgtcccctggcaag

SEQ ID NO: 26 - DNA, 642 bp, Nucleic acid sequence encoding '996 light chain
gacatccagatgactcagtccccctctagcctgagcgctagcgtgggcgacagggtgaccatcacctgccaggccagccaggacatcagcaccttcctgaactggtaccagcagaagcccggcaaggcccccaaactgctgatctacgacgcctcaaacctcgagaccggcgtgcctagcaggtttagcggcagcggcagcggcaccgacttcaccttcaccatcagcagcctgcagcccgaggatatcgccacctactactgccagcaggacagcatcctgcccatcaccttcggcggaggcaccaaggtggagattaagcgtacggtggccgcccccagcgtgttcatcttcccccccagcgatgagcagctgaagagcggcaccgccagcgtggtgtgtctgctgaacaacttctacccccgggaggccaaggtgcagtggaaggtggacaatgccctgcagagcggcaacagccaggagagcgtgaccgagcaggacagcaaggactccacctacagcctgagcagcaccctgaccctgagcaaggccgactacgagaagcacaaggtgtacgcctgtgaggtgacccaccagggcctgtccagccccgtgaccaagagcttcaaccggggcgagtgc

SEQ ID NO: 27 - protein, 449 aa, Artificial Sequence
  Amino acid sequence identified using molecular biology techniques
QLQLQESGPGLVKPSETLSLTCTVSGGSISSSSYYWGWIRQPPGKGLEWIGSIHYSGSTYYNPPLESRVTISVDTSKNQFSLKLSSVTAADTAVYYCAREGGPRHGWSWGQGTLVTVSSASTKGPSVFPLAPSSKSTSGGTAALGCLVKDYFPEPVTVSWNSGALTSGVHTFPAVLQSSGLYSLSSVVTVPSSSLGTQTYICNVNHKPSNTKVDKKVEPKSCDKTHTCPPCPAPELAGAPSVFLFPPKPKDTLMISRTPEVTCVVVDVSHEDPEVKFNWYVDGVEVHNAKTKPREEQYNSTYRVVSVLTVLHQDWLNGKEYKCKVSNKALPAPIEKTISKAKGQPREPQVYTLPPSRDELTKNQVSLTCLVKGFYPSDIAVEWESNGQPENNYKTTPPVLDSDGSFFLYSKLTVDKSRWQQGNVFSCSVMHEALHNHYTQKSLSLSPGK

SEQ ID NO: 28 - protein, 214 aa, Artificial Sequence
  Amino acid sequence identified using molecular biology techniques
DIQMTQSPSSLSASVGDRVTITCQASHDISNFLNWYQQKPGKAPKLLIYDTSNLETGVPSRFSGSGSGTDFTFTISSLQPEDIATYYCQQDSILPITFGGGTKVEIKRTVAAPSVFIFPPSDEQLKSGTASVVCLLNNFYPREAKVQWKVDNALQSGNSQESVTEQDSKDSTYSLSSTLTLSKADYEKHKVYACEVTHQGLSSPVTKSFNRGEC

SEQ ID NO: 29 - protein, 119 aa, Artificial Sequence
  Amino acid sequence identified using molecular biology techniques
QLQLQESGPGLVKPSETLSLTCTVSGGSISSSSYYWGWIRQPPGKGLEWIGSIHYSGSTYYNPPLESRVTISVDTSKNQFSLKLSSVTAADTAVYYCAREGGPRHGWSWGQGTLVTVSS

SEQ ID NO: 30 - protein, 107 aa, Artificial Sequence
  Amino acid sequence identified using molecular biology techniques
DIQMTQSPSSLSASVGDRVTITCQASHDISNFLNWYQQKPGKAPKLLIYDTSNLETGVPSRFSGSGSGTDFTFTISSLQPEDIATYYCQQDSILPITFGGGTKVEIK

SEQ ID NO: 31 - protein, 7 aa, Artificial Sequence
  Amino acid sequence identified using molecular biology techniques
SSSYYWG

SEQ ID NO: 32 - protein, 16 aa, Artificial Sequence
  Amino acid sequence identified using molecular biology techniques
SIHYSGSTYYNPPLES

SEQ ID NO: 33 - protein, 9 aa, Artificial Sequence
  Amino acid sequence identified using molecular biology techniques
EGGPRHGWS

SEQ ID NO: 34 - protein, 11 aa, Artificial Sequence
  Amino acid sequence identified using molecular biology techniques
QASHDISNFLN

SEQ ID NO: 35 - protein, 7 aa, Artificial Sequence
  Amino acid sequence identified using molecular biology techniques
DTSNLET

SEQ ID NO: 36 - protein, 9 aa, Artificial Sequence
  Amino acid sequence identified using molecular biology techniques
QQDSILPIT

SEQ ID NO: 37 - DNA, 1347 bp, Nucleic acid sequence encoding '999 heavy chain
cagctccagctgcaggagagcggcccaggcctggtgaaacccagcgagaccctgagcctgacctgcaccgtgagcggaggcagcatcagctccagcagctactactggggctggattaggcagcctcccggcaagggcctggagtggatcggaagcatccactacagcggcagcacctactacaacccacccctggagagcagggtgaccatcagcgtggacaccagcaagaaccagttcagcctgaagctgagcagcgtcacagcagccgacaccgccgtgtactattgcgccagggagggcggacccaggcacggctggagctggggccagggcaccctggtgaccgtgagcagcgcaagcaccaagggccccagcgtgttccccctggcccccagcagcaagagcaccagcggcggcacagccgccctgggctgcctggtgaaggactacttccccgagcccgtgaccgtgtcctggaacagcggagccctgaccagcggcgtgcacaccttccccgccgtgctgcagagcagcggcctgtacagcctgagcagcgtggtgaccgtgcccagcagcagcctgggcacccagacctacatctgtaacgtgaaccacaagcccagcaacaccaaggtggacaagaaggtggagcccaagagctgtgacaagacccacacctgccccccctgccctgcccccgagctggccggagcccccagcgtgttcctgttcccccccaagcctaaggacaccctgatgatcagcagaacccccgaggtgacctgtgtggtggtggatgtgagccacgaggaccctgaggtgaagttcaactggtacgtggacggcgtggaggtgcacaatgccaagaccaagcccagggaggagcagtacaacagcacctaccgggtggtgtccgtgctgaccgtgctgcaccaggattggctgaacggcaaggagtacaagtgtaaggtgtccaacaaggccctgcctgcccctatcgagaaaaccatcagcaaggccaagggccagcccagagagccccaggtgtacaccctgccccctagcagagatgagctgaccaagaaccaggtgtccctgacctgcctggtgaagggcttctaccccagcgacatcgccgtggagtgggagagcaacggccagcccgagaacaactacaagaccaccccccctgtgctggacagcgatggcagcttcttcctgtacagcaagctgaccgtggacaagagcagatggcagcagggcaacgtgttcagctgctccgtgatgcacgaggccctgcacaatcactacacccagaagagcctgagcctgtcccctggcaag

SEQ ID NO: 38 - DNA, 642 bp, Nucleic acid sequence encoding '999 light chain
gacatccagatgactcagtccccctctagcctgagcgctagcgtgggcgacagggtgaccatcacctgccaggccagccacgacatcagcaacttcctgaactggtaccagcagaagcccggcaaggcccccaaactgctgatctacgacacctcaaacctcgagaccggcgtgcctagcaggtttagcggcagcggcagcggcaccgacttcaccttcaccatcagcagcctgcagcccgaggatatcgccacctactactgccagcaggacagcatcctgcccatcaccttcggcggaggcaccaaggtggagattaagcgtacggtggccgcccccagcgtgttcatcttcccccccagcgatgagcagctgaagagcggcaccgccagcgtggtgtgtctgctgaacaacttctacccccgggaggccaaggtgcagtggaaggtggacaatgccctgcagagcggcaacagccaggagagcgtgaccgagcaggacagcaaggactccacctacagcctgagcagcaccctgaccctgagcaaggccgactacgagaagcacaaggtgtacgcctgtgaggtgacccaccagggcctgtccagccccgtgaccaagagcttcaaccggggcgagtgc

SEQ ID NO: 39 - protein, 11 aa, Artificial Sequence
  Amino acid sequence identified using molecular biology techniques
MISCGSPPPIL

SEQ ID NO: 40 - protein, 17 aa, Artificial Sequence
  Amino acid sequence identified using molecular biology techniques
MISCGSPPPILNGRISY

SEQ ID NO: 41 - protein, 8 aa, Artificial Sequence
  Amino acid sequence identified using molecular biology techniques
YSTPIAVG

SEQ ID NO: 42 - protein, 9 aa, Artificial Sequence
  Amino acid sequence identified using molecular biology techniques
YSTPIAVGT

SEQ ID NO: 43 - protein, 18 aa, Artificial Sequence
  Amino acid sequence identified using molecular biology techniques
YSTPIAVGTVIRYSCSGT

SEQ ID NO: 44 - protein, 10 aa, Artificial Sequence
  Amino acid sequence identified using molecular biology techniques
TVIRYSCSGT

SEQ ID NO: 45 - protein, 11 aa, Artificial Sequence
  Amino acid sequence identified using molecular biology techniques
TVIRYSCSGTF

SEQ ID NO: 46 - protein, 9 aa, Artificial Sequence
  Amino acid sequence identified using molecular biology techniques
VIRYSCSGT

SEQ ID NO: 47 - protein, 8 aa, Artificial Sequence
  Amino acid sequence identified using molecular biology techniques
FRLIGEKS

SEQ ID NO: 48 - protein, 9 aa, Artificial Sequence
  Amino acid sequence identified using molecular biology techniques
FRLIGEKSL

SEQ ID NO: 49 - protein, 10 aa, Artificial Sequence
  Amino acid sequence identified using molecular biology techniques
FRLIGEKSLL

SEQ ID NO: 50 - protein, 8 aa, Artificial Sequence
  Amino acid sequence identified using molecular biology techniques
RLIGEKSL

SEQ ID NO: 51 - protein, 9 aa, Artificial Sequence
  Amino acid sequence identified using molecular biology techniques
RLIGEKSLL

SEQ ID NO: 52 - protein, 7 aa, Artificial Sequence
  Amino acid sequence identified using molecular biology techniques
IGEKSLL

SEQ ID NO: 53 - protein, 21 aa, Artificial Sequence
  Amino acid sequence identified using molecular biology techniques
GEKSLLCITKDKVDGTWDKPA

SEQ ID NO: 54 - protein, 10 aa, Artificial Sequence
  Amino acid sequence identified using molecular biology techniques
CITKDKVDGT

SEQ ID NO: 55 - protein, 20 aa, Artificial Sequence
  Amino acid sequence identified using molecular biology techniques
CITKDKVDGTWDKPAPKCEY

SEQ ID NO: 56 - protein, 15 aa, Artificial Sequence
  Amino acid sequence identified using molecular biology techniques
KVDGTWDKPAPKCEY

SEQ ID NO: 57 - protein, 10 aa, Artificial Sequence
  Amino acid sequence identified using molecular biology techniques
WDKPAPKCEY

SEQ ID NO: 58 - protein, 31 aa, Artificial Sequence
  Amino acid sequence identified using molecular biology techniques
FNKYSSCPEPIVPGGYKIRGSTPYRHGDSVT

SEQ ID NO: 59 - protein, 32 aa, Artificial Sequence
  Amino acid sequence identified using molecular biology techniques
FNKYSSCPEPIVPGGYKIRGSTPYRHGDSVTF

SEQ ID NO: 60 - protein, 27 aa, Artificial Sequence
  Amino acid sequence identified using molecular biology techniques
SSCPEPIVPGGYKIRGSTPYRHGDSVT

SEQ ID NO: 61 - protein, 16 aa, Artificial Sequence
  Amino acid sequence identified using molecular biology techniques
YKIRGSTPYRHGDSVT

SEQ ID NO: 62 - protein, 17 aa, Artificial Sequence
  Amino acid sequence identified using molecular biology techniques
YKIRGSTPYRHGDSVTF

SEQ ID NO: 63 - protein, 15 aa, Artificial Sequence
  Amino acid sequence identified using molecular biology techniques
KIRGSTPYRHGDSVT

SEQ ID NO: 64 - protein, 16 aa, Artificial Sequence
  Amino acid sequence identified using molecular biology techniques
KIRGSTPYRHGDSVTF

SEQ ID NO: 65 - protein, 7 aa, Artificial Sequence
  Amino acid sequence identified using molecular biology techniques
FACKTNF

SEQ ID NO: 66 - protein, 9 aa, Artificial Sequence
  Amino acid sequence identified using molecular biology techniques
SMNGNKSVW

SEQ ID NO: 67 - protein, 10 aa, Artificial Sequence
  Amino acid sequence identified using molecular biology techniques
SMNGNKSVWC

SEQ ID NO: 68 - protein, 12 aa, Artificial Sequence
  Amino acid sequence identified using molecular biology techniques
SMNGNKSVWCQA

SEQ ID NO: 69 - protein, 15 aa, Artificial Sequence
  Amino acid sequence identified using molecular biology techniques
SMNGNKSVWCQANNM

SEQ ID NO: 70 - protein, 21 aa, Artificial Sequence
  Amino acid sequence identified using molecular biology techniques
SMNGNKSVWCQANNMWGPTRL

SEQ ID NO: 71 - protein, 24 aa, Artificial Sequence
  Amino acid sequence identified using molecular biology techniques
SMNGNKSVWCQANNMWGPTRLPTC

SEQ ID NO: 72 - protein, 9 aa, Artificial Sequence
  Amino acid sequence identified using molecular biology techniques
NNMWGPTRL

SEQ ID NO: 73 - protein, 13 aa, Artificial Sequence
  Amino acid sequence identified using molecular biology techniques
NNMWGPTRLPTCV

SEQ ID NO: 74 - protein, 7 aa, Artificial Sequence
  Amino acid sequence identified using molecular biology techniques
VSVFPLE